European Patent Specification EP 3 926 052 B1, published January 14, 2026. Title: Oligonucleotide conjugate with high hybridization performance and use thereof. Applicant: Daan Gene Co., Ltd. Of Sun Yat-Sen University. The sequence listing filed with the application follows.

SEQUENCE LISTING (14 sequences)

SEQ ID NO: 1 - DNA, 23 bp, Artificial sequence
  Primer
gtagatctccgtttctattgctt

SEQ ID NO: 2 - DNA, 16 bp, Artificial sequence
  Primer
cctctagcgctgcgaa

SEQ ID NO: 3 - DNA, 29 bp, Artificial sequence
  Probe
tagcactatcaagccttccctttatacgc

SEQ ID NO: 4 - DNA, 21 bp, Artificial sequence
  Probe
agcactatcaagccttccctt

SEQ ID NO: 5 - DNA, 21 bp, Artificial sequence
  Probe
tcaagccttccctttatacgc

SEQ ID NO: 6 - DNA, 20 bp, Artificial sequence
  Probe
agcactatcaagccttccct

SEQ ID NO: 7 - DNA, 20 bp, Artificial sequence
  Probe
caagccttccctttatacgc

SEQ ID NO: 8 - DNA, 18 bp, Artificial sequence
  Probe
tcaagccttccctttata

SEQ ID NO: 9 - DNA, 18 bp, Artificial sequence
  Probe
aagccttccctttatacg

SEQ ID NO: 10 - DNA, 17 bp, Artificial sequence
  Probe
cactatcaagccttccc

SEQ ID NO: 11 - DNA, 21 bp, Artificial sequence
  Probe
agcactatcaagccttccctt

SEQ ID NO: 12 - DNA, 21 bp, Artificial sequence
  Probe
tcaagccttccctttatacgc

SEQ ID NO: 13 - DNA, 20 bp, Artificial sequence
  Probe
agcactatcaagccttccct

SEQ ID NO: 14 - DNA, 20 bp, Artificial sequence
  Probe
caagccttccctttatacgc